European Patent Application EP 4 289 953 A1, published December 13, 2023. Title: DOUBLE-STRANDED NUCLEIC ACID MOLECULE FOR TREATING PROLIFERATIVE VITREORETINOPATHY AND USE THEREOF. Applicant: Ractigen Therapeutics. Application EP22749094.3. The sequence listing filed with the application follows.

SEQUENCE LISTING (511 sequences)

SEQ ID NO: 1 - DNA, 21 bp, Artificial Sequence
  Primer sequence
atcaccatcttccaggagcga

SEQ ID NO: 2 - DNA, 21 bp, Artificial Sequence
  Primer sequence
ttctccatggtggtgaagacg

SEQ ID NO: 3 - DNA, 20 bp, Artificial Sequence
  Primer sequence
ggaagaccatgtggacctgt

SEQ ID NO: 4 - DNA, 20 bp, Artificial Sequence
  Primer sequence
ggattagggcttcctcttgg

SEQ ID NO: 5 - DNA, 92 bp, Homo sapiens
ggctatgtggggagtattcaggagacagacaactcactcgtcaaatcctccccttcctggccaacaaagctgctgcaaccacagggatttct

SEQ ID NO: 6 - DNA, 86 bp, Homo sapiens
ggtagtctctccaattccctccttcccggaagcatgtgacaatcaacaactttgtatacttaagttcagtggacctcaatttcctc

SEQ ID NO: 7 - DNA, 35 bp, Homo sapiens
ctttgttggggtgtctaggtgctccaggtgcttct

SEQ ID NO: 8 - DNA, 51 bp, Homo sapiens
ttctgggagaggtgacctagtgagggatcagtgggaatagaggtgatattg

SEQ ID NO: 9 - DNA, 30 bp, Homo sapiens
aggtgatattgtggggcttttctggaaatt

SEQ ID NO: 10 - DNA, 38 bp, Homo sapiens
attaatgtcatcctcctgatcttttcagctgcattggg

SEQ ID NO: 11 - DNA, 40 bp, Homo sapiens
tctaacagtgctgtgtcctcctggagagtgccaactcatt

SEQ ID NO: 12 - DNA, 66 bp, Homo sapiens
gtgccaactcattctccaagtaaaaaaagccagatttgtggctcacttcgtggggaaatgtgtcca

SEQ ID NO: 13 - DNA, 21 bp, Artificial Sequence
  Oligonucleotide sequence
ucguggggaaauguguccatt

SEQ ID NO: 14 - DNA, 21 bp, Artificial Sequence
  Oligonucleotide sequence
uggacacauuuccccacgatt

SEQ ID NO: 15 - DNA, 21 bp, Artificial Sequence
  Oligonucleotide sequence
uucguggggaaaugugucctt

SEQ ID NO: 16 - DNA, 21 bp, Artificial Sequence
  Oligonucleotide sequence
ggacacauuuccccacgaatt

SEQ ID NO: 17 - DNA, 21 bp, Artificial Sequence
  Oligonucleotide sequence
cuucguggggaaauguguctt

SEQ ID NO: 18 - DNA, 21 bp, Artificial Sequence
  Oligonucleotide sequence
gacacauuuccccacgaagtt

SEQ ID NO: 19 - DNA, 21 bp, Artificial Sequence
  Oligonucleotide sequence
acuucguggggaaaugugutt

SEQ ID NO: 20 - DNA, 21 bp, Artificial Sequence
  Oligonucleotide sequence
acacauuuccccacgaagutt

SEQ ID NO: 21 - DNA, 21 bp, Artificial Sequence
  Oligonucleotide sequence
cacuucguggggaaaugugtt

SEQ ID NO: 22 - DNA, 21 bp, Artificial Sequence
  Oligonucleotide sequence
cacauuuccccacgaagugtt

SEQ ID NO: 23 - DNA, 21 bp, Artificial Sequence
  Oligonucleotide sequence
ucacuucguggggaaaugutt

SEQ ID NO: 24 - DNA, 21 bp, Artificial Sequence
  Oligonucleotide sequence
acauuuccccacgaagugatt

SEQ ID NO: 25 - DNA, 21 bp, Artificial Sequence
  Oligonucleotide sequence
cucacuucguggggaaaugtt

SEQ ID NO: 26 - DNA, 21 bp, Artificial Sequence
  Oligonucleotide sequence
cauuuccccacgaagugagtt

SEQ ID NO: 27 - DNA, 21 bp, Artificial Sequence
  Oligonucleotide sequence
gcucacuucguggggaaautt

SEQ ID NO: 28 - DNA, 21 bp, Artificial Sequence
  Oligonucleotide sequence
auuuccccacgaagugagctt

SEQ ID NO: 29 - DNA, 21 bp, Artificial Sequence
  Oligonucleotide sequence
ggcucacuucguggggaaatt

SEQ ID NO: 30 - DNA, 21 bp, Artificial Sequence
  Oligonucleotide sequence
uuuccccacgaagugagcctt

SEQ ID NO: 31 - DNA, 21 bp, Artificial Sequence
  Oligonucleotide sequence
uggcucacuucguggggaatt

SEQ ID NO: 32 - DNA, 21 bp, Artificial Sequence
  Oligonucleotide sequence
uuccccacgaagugagccatt

SEQ ID NO: 33 - DNA, 21 bp, Artificial Sequence
  Oligonucleotide sequence
guggcucacuucguggggatt

SEQ ID NO: 34 - DNA, 21 bp, Artificial Sequence
  Oligonucleotide sequence
uccccacgaagugagccactt

SEQ ID NO: 35 - DNA, 21 bp, Artificial Sequence
  Oligonucleotide sequence
uguggcucacuucguggggtt

SEQ ID NO: 36 - DNA, 21 bp, Artificial Sequence
  Oligonucleotide sequence
ccccacgaagugagccacatt

SEQ ID NO: 37 - DNA, 21 bp, Artificial Sequence
  Oligonucleotide sequence
uuuguggcucacuucguggtt

SEQ ID NO: 38 - DNA, 21 bp, Artificial Sequence
  Oligonucleotide sequence
ccacgaagugagccacaaatt

SEQ ID NO: 39 - DNA, 21 bp, Artificial Sequence
  Oligonucleotide sequence
auuuguggcucacuucgugtt

SEQ ID NO: 40 - DNA, 21 bp, Artificial Sequence
  Oligonucleotide sequence
cacgaagugagccacaaautt

SEQ ID NO: 41 - DNA, 21 bp, Artificial Sequence
  Oligonucleotide sequence
gauuuguggcucacuucgutt

SEQ ID NO: 42 - DNA, 21 bp, Artificial Sequence
  Oligonucleotide sequence
acgaagugagccacaaauctt

SEQ ID NO: 43 - DNA, 21 bp, Artificial Sequence
  Oligonucleotide sequence
agauuuguggcucacuucgtt

SEQ ID NO: 44 - DNA, 21 bp, Artificial Sequence
  Oligonucleotide sequence
cgaagugagccacaaaucutt

SEQ ID NO: 45 - DNA, 21 bp, Artificial Sequence
  Oligonucleotide sequence
cagauuuguggcucacuuctt

SEQ ID NO: 46 - DNA, 21 bp, Artificial Sequence
  Oligonucleotide sequence
gaagugagccacaaaucugtt

SEQ ID NO: 47 - DNA, 21 bp, Artificial Sequence
  Oligonucleotide sequence
ccagauuuguggcucacuutt

SEQ ID NO: 48 - DNA, 21 bp, Artificial Sequence
  Oligonucleotide sequence
aagugagccacaaaucuggtt

SEQ ID NO: 49 - DNA, 21 bp, Artificial Sequence
  Oligonucleotide sequence
gccagauuuguggcucacutt

SEQ ID NO: 50 - DNA, 21 bp, Artificial Sequence
  Oligonucleotide sequence
agugagccacaaaucuggctt

SEQ ID NO: 51 - DNA, 21 bp, Artificial Sequence
  Oligonucleotide sequence
agccagauuuguggcucactt

SEQ ID NO: 52 - DNA, 21 bp, Artificial Sequence
  Oligonucleotide sequence
gugagccacaaaucuggcutt

SEQ ID NO: 53 - DNA, 21 bp, Artificial Sequence
  Oligonucleotide sequence
aagccagauuuguggcucatt

SEQ ID NO: 54 - DNA, 21 bp, Artificial Sequence
  Oligonucleotide sequence
ugagccacaaaucuggcuutt

SEQ ID NO: 55 - DNA, 21 bp, Artificial Sequence
  Oligonucleotide sequence
aaagccagauuuguggcuctt

SEQ ID NO: 56 - DNA, 21 bp, Artificial Sequence
  Oligonucleotide sequence
gagccacaaaucuggcuuutt

SEQ ID NO: 57 - DNA, 21 bp, Artificial Sequence
  Oligonucleotide sequence
aaaagccagauuuguggcutt

SEQ ID NO: 58 - DNA, 21 bp, Artificial Sequence
  Oligonucleotide sequence
agccacaaaucuggcuuuutt

SEQ ID NO: 59 - DNA, 21 bp, Artificial Sequence
  Oligonucleotide sequence
caacucauucuccaaguaatt

SEQ ID NO: 60 - DNA, 21 bp, Artificial Sequence
  Oligonucleotide sequence
uuacuuggagaaugaguugtt

SEQ ID NO: 61 - DNA, 21 bp, Artificial Sequence
  Oligonucleotide sequence
ccaacucauucuccaaguatt

SEQ ID NO: 62 - DNA, 21 bp, Artificial Sequence
  Oligonucleotide sequence
uacuuggagaaugaguuggtt

SEQ ID NO: 63 - DNA, 21 bp, Artificial Sequence
  Oligonucleotide sequence
gccaacucauucuccaagutt

SEQ ID NO: 64 - DNA, 21 bp, Artificial Sequence
  Oligonucleotide sequence
acuuggagaaugaguuggctt

SEQ ID NO: 65 - DNA, 21 bp, Artificial Sequence
  Oligonucleotide sequence
ugccaacucauucuccaagtt

SEQ ID NO: 66 - DNA, 21 bp, Artificial Sequence
  Oligonucleotide sequence
cuuggagaaugaguuggcatt

SEQ ID NO: 67 - DNA, 21 bp, Artificial Sequence
  Oligonucleotide sequence
gugccaacucauucuccaatt

SEQ ID NO: 68 - DNA, 21 bp, Artificial Sequence
  Oligonucleotide sequence
uuggagaaugaguuggcactt

SEQ ID NO: 69 - DNA, 21 bp, Artificial Sequence
  Oligonucleotide sequence
uggagagugccaacucauutt

SEQ ID NO: 70 - DNA, 21 bp, Artificial Sequence
  Oligonucleotide sequence
aaugaguuggcacucuccatt

SEQ ID NO: 71 - DNA, 21 bp, Artificial Sequence
  Oligonucleotide sequence
cuggagagugccaacucautt

SEQ ID NO: 72 - DNA, 21 bp, Artificial Sequence
  Oligonucleotide sequence
augaguuggcacucuccagtt

SEQ ID NO: 73 - DNA, 21 bp, Artificial Sequence
  Oligonucleotide sequence
ccuggagagugccaacucatt

SEQ ID NO: 74 - DNA, 21 bp, Artificial Sequence
  Oligonucleotide sequence
ugaguuggcacucuccaggtt

SEQ ID NO: 75 - DNA, 21 bp, Artificial Sequence
  Oligonucleotide sequence
uccuggagagugccaacuctt

SEQ ID NO: 76 - DNA, 21 bp, Artificial Sequence
  Oligonucleotide sequence
gaguuggcacucuccaggatt

SEQ ID NO: 77 - DNA, 21 bp, Artificial Sequence
  Oligonucleotide sequence
cuccuggagagugccaacutt

SEQ ID NO: 78 - DNA, 21 bp, Artificial Sequence
  Oligonucleotide sequence
aguuggcacucuccaggagtt

SEQ ID NO: 79 - DNA, 21 bp, Artificial Sequence
  Oligonucleotide sequence
ccuccuggagagugccaactt

SEQ ID NO: 80 - DNA, 21 bp, Artificial Sequence
  Oligonucleotide sequence
guuggcacucuccaggaggtt

SEQ ID NO: 81 - DNA, 21 bp, Artificial Sequence
  Oligonucleotide sequence
uccuccuggagagugccaatt

SEQ ID NO: 82 - DNA, 21 bp, Artificial Sequence
  Oligonucleotide sequence
uuggcacucuccaggaggatt

SEQ ID NO: 83 - DNA, 21 bp, Artificial Sequence
  Oligonucleotide sequence
guccuccuggagagugccatt

SEQ ID NO: 84 - DNA, 21 bp, Artificial Sequence
  Oligonucleotide sequence
uggcacucuccaggaggactt

SEQ ID NO: 85 - DNA, 21 bp, Artificial Sequence
  Oligonucleotide sequence
uguguccuccuggagagugtt

SEQ ID NO: 86 - DNA, 21 bp, Artificial Sequence
  Oligonucleotide sequence
cacucuccaggaggacacatt

SEQ ID NO: 87 - DNA, 21 bp, Artificial Sequence
  Oligonucleotide sequence
cuguguccuccuggagagutt

SEQ ID NO: 88 - DNA, 21 bp, Artificial Sequence
  Oligonucleotide sequence
acucuccaggaggacacagtt

SEQ ID NO: 89 - DNA, 21 bp, Artificial Sequence
  Oligonucleotide sequence
gcuguguccuccuggagagtt

SEQ ID NO: 90 - DNA, 21 bp, Artificial Sequence
  Oligonucleotide sequence
cucuccaggaggacacagctt

SEQ ID NO: 91 - DNA, 21 bp, Artificial Sequence
  Oligonucleotide sequence
ugcuguguccuccuggagatt

SEQ ID NO: 92 - DNA, 21 bp, Artificial Sequence
  Oligonucleotide sequence
ucuccaggaggacacagcatt

SEQ ID NO: 93 - DNA, 21 bp, Artificial Sequence
  Oligonucleotide sequence
gugcuguguccuccuggagtt

SEQ ID NO: 94 - DNA, 21 bp, Artificial Sequence
  Oligonucleotide sequence
cuccaggaggacacagcactt

SEQ ID NO: 95 - DNA, 21 bp, Artificial Sequence
  Oligonucleotide sequence
agugcuguguccuccuggatt

SEQ ID NO: 96 - DNA, 21 bp, Artificial Sequence
  Oligonucleotide sequence
uccaggaggacacagcacutt

SEQ ID NO: 97 - DNA, 21 bp, Artificial Sequence
  Oligonucleotide sequence
acagugcuguguccuccugtt

SEQ ID NO: 98 - DNA, 21 bp, Artificial Sequence
  Oligonucleotide sequence
caggaggacacagcacugutt

SEQ ID NO: 99 - DNA, 21 bp, Artificial Sequence
  Oligonucleotide sequence
aacagugcuguguccuccutt

SEQ ID NO: 100 - DNA, 21 bp, Artificial Sequence
  Oligonucleotide sequence
aggaggacacagcacuguutt

SEQ ID NO: 101 - DNA, 21 bp, Artificial Sequence
  Oligonucleotide sequence
uaacagugcuguguccucctt

SEQ ID NO: 102 - DNA, 21 bp, Artificial Sequence
  Oligonucleotide sequence
ggaggacacagcacuguuatt

SEQ ID NO: 103 - DNA, 21 bp, Artificial Sequence
  Oligonucleotide sequence
cuaacagugcuguguccuctt

SEQ ID NO: 104 - DNA, 21 bp, Artificial Sequence
  Oligonucleotide sequence
gaggacacagcacuguuagtt

SEQ ID NO: 105 - DNA, 21 bp, Artificial Sequence
  Oligonucleotide sequence
ucuaacagugcuguguccutt

SEQ ID NO: 106 - DNA, 21 bp, Artificial Sequence
  Oligonucleotide sequence
aggacacagcacuguuagatt

SEQ ID NO: 107 - DNA, 21 bp, Artificial Sequence
  Oligonucleotide sequence
ucuuuucagcugcauugggtt

SEQ ID NO: 108 - DNA, 21 bp, Artificial Sequence
  Oligonucleotide sequence
cccaaugcagcugaaaagatt

SEQ ID NO: 109 - DNA, 21 bp, Artificial Sequence
  Oligonucleotide sequence
aucuuuucagcugcauuggtt

SEQ ID NO: 110 - DNA, 21 bp, Artificial Sequence
  Oligonucleotide sequence
ccaaugcagcugaaaagautt

SEQ ID NO: 111 - DNA, 21 bp, Artificial Sequence
  Oligonucleotide sequence
gaucuuuucagcugcauugtt

SEQ ID NO: 112 - DNA, 21 bp, Artificial Sequence
  Oligonucleotide sequence
caaugcagcugaaaagauctt

SEQ ID NO: 113 - DNA, 21 bp, Artificial Sequence
  Oligonucleotide sequence
ugaucuuuucagcugcauutt

SEQ ID NO: 114 - DNA, 21 bp, Artificial Sequence
  Oligonucleotide sequence
aaugcagcugaaaagaucatt

SEQ ID NO: 115 - DNA, 21 bp, Artificial Sequence
  Oligonucleotide sequence
cugaucuuuucagcugcautt

SEQ ID NO: 116 - DNA, 21 bp, Artificial Sequence
  Oligonucleotide sequence
augcagcugaaaagaucagtt

SEQ ID NO: 117 - DNA, 21 bp, Artificial Sequence
  Oligonucleotide sequence
ccugaucuuuucagcugcatt

SEQ ID NO: 118 - DNA, 21 bp, Artificial Sequence
  Oligonucleotide sequence
ugcagcugaaaagaucaggtt

SEQ ID NO: 119 - DNA, 21 bp, Artificial Sequence
  Oligonucleotide sequence
uccugaucuuuucagcugctt

SEQ ID NO: 120 - DNA, 21 bp, Artificial Sequence
  Oligonucleotide sequence
gcagcugaaaagaucaggatt

SEQ ID NO: 121 - DNA, 21 bp, Artificial Sequence
  Oligonucleotide sequence
cuccugaucuuuucagcugtt

SEQ ID NO: 122 - DNA, 21 bp, Artificial Sequence
  Oligonucleotide sequence
cagcugaaaagaucaggagtt

SEQ ID NO: 123 - DNA, 21 bp, Artificial Sequence
  Oligonucleotide sequence
ccuccugaucuuuucagcutt

SEQ ID NO: 124 - DNA, 21 bp, Artificial Sequence
  Oligonucleotide sequence
agcugaaaagaucaggaggtt

SEQ ID NO: 125 - DNA, 21 bp, Artificial Sequence
  Oligonucleotide sequence
uccuccugaucuuuucagctt

SEQ ID NO: 126 - DNA, 21 bp, Artificial Sequence
  Oligonucleotide sequence
gcugaaaagaucaggaggatt

SEQ ID NO: 127 - DNA, 21 bp, Artificial Sequence
  Oligonucleotide sequence
auccuccugaucuuuucagtt

SEQ ID NO: 128 - DNA, 21 bp, Artificial Sequence
  Oligonucleotide sequence
cugaaaagaucaggaggautt

SEQ ID NO: 129 - DNA, 21 bp, Artificial Sequence
  Oligonucleotide sequence
cauccuccugaucuuuucatt

SEQ ID NO: 130 - DNA, 21 bp, Artificial Sequence
  Oligonucleotide sequence
ugaaaagaucaggaggaugtt

SEQ ID NO: 131 - DNA, 21 bp, Artificial Sequence
  Oligonucleotide sequence
ucauccuccugaucuuuuctt

SEQ ID NO: 132 - DNA, 21 bp, Artificial Sequence
  Oligonucleotide sequence
gaaaagaucaggaggaugatt

SEQ ID NO: 133 - DNA, 21 bp, Artificial Sequence
  Oligonucleotide sequence
gucauccuccugaucuuuutt

SEQ ID NO: 134 - DNA, 21 bp, Artificial Sequence
  Oligonucleotide sequence
aaaagaucaggaggaugactt

SEQ ID NO: 135 - DNA, 21 bp, Artificial Sequence
  Oligonucleotide sequence
ugucauccuccugaucuuutt

SEQ ID NO: 136 - DNA, 21 bp, Artificial Sequence
  Oligonucleotide sequence
aaagaucaggaggaugacatt

SEQ ID NO: 137 - DNA, 21 bp, Artificial Sequence
  Oligonucleotide sequence
augucauccuccugaucuutt

SEQ ID NO: 138 - DNA, 21 bp, Artificial Sequence
  Oligonucleotide sequence
aagaucaggaggaugacautt

SEQ ID NO: 139 - DNA, 21 bp, Artificial Sequence
  Oligonucleotide sequence
aaugucauccuccugaucutt

SEQ ID NO: 140 - DNA, 21 bp, Artificial Sequence
  Oligonucleotide sequence
agaucaggaggaugacauutt

SEQ ID NO: 141 - DNA, 21 bp, Artificial Sequence
  Oligonucleotide sequence
uaaugucauccuccugauctt

SEQ ID NO: 142 - DNA, 21 bp, Artificial Sequence
  Oligonucleotide sequence
gaucaggaggaugacauuatt

SEQ ID NO: 143 - DNA, 21 bp, Artificial Sequence
  Oligonucleotide sequence
uuaaugucauccuccugautt

SEQ ID NO: 144 - DNA, 21 bp, Artificial Sequence
  Oligonucleotide sequence
aucaggaggaugacauuaatt

SEQ ID NO: 145 - DNA, 21 bp, Artificial Sequence
  Oligonucleotide sequence
auuaaugucauccuccugatt

SEQ ID NO: 146 - DNA, 21 bp, Artificial Sequence
  Oligonucleotide sequence
ucaggaggaugacauuaautt

SEQ ID NO: 147 - DNA, 21 bp, Artificial Sequence
  Oligonucleotide sequence
uggggcuuuucuggaaauutt

SEQ ID NO: 148 - DNA, 21 bp, Artificial Sequence
  Oligonucleotide sequence
aauuuccagaaaagccccatt

SEQ ID NO: 149 - DNA, 21 bp, Artificial Sequence
  Oligonucleotide sequence
guggggcuuuucuggaaautt

SEQ ID NO: 150 - DNA, 21 bp, Artificial Sequence
  Oligonucleotide sequence
auuuccagaaaagccccactt

SEQ ID NO: 151 - DNA, 21 bp, Artificial Sequence
  Oligonucleotide sequence
uguggggcuuuucuggaaatt

SEQ ID NO: 152 - DNA, 21 bp, Artificial Sequence
  Oligonucleotide sequence
uuuccagaaaagccccacatt

SEQ ID NO: 153 - DNA, 21 bp, Artificial Sequence
  Oligonucleotide sequence
uuguggggcuuuucuggaatt

SEQ ID NO: 154 - DNA, 21 bp, Artificial Sequence
  Oligonucleotide sequence
uuccagaaaagccccacaatt

SEQ ID NO: 155 - DNA, 21 bp, Artificial Sequence
  Oligonucleotide sequence
auuguggggcuuuucuggatt

SEQ ID NO: 156 - DNA, 21 bp, Artificial Sequence
  Oligonucleotide sequence
uccagaaaagccccacaautt

SEQ ID NO: 157 - DNA, 21 bp, Artificial Sequence
  Oligonucleotide sequence
uauuguggggcuuuucuggtt

SEQ ID NO: 158 - DNA, 21 bp, Artificial Sequence
  Oligonucleotide sequence
ccagaaaagccccacaauatt

SEQ ID NO: 159 - DNA, 21 bp, Artificial Sequence
  Oligonucleotide sequence
auauuguggggcuuuucugtt

SEQ ID NO: 160 - DNA, 21 bp, Artificial Sequence
  Oligonucleotide sequence
cagaaaagccccacaauautt

SEQ ID NO: 161 - DNA, 21 bp, Artificial Sequence
  Oligonucleotide sequence
gauauuguggggcuuuucutt

SEQ ID NO: 162 - DNA, 21 bp, Artificial Sequence
  Oligonucleotide sequence
agaaaagccccacaauauctt

SEQ ID NO: 163 - DNA, 21 bp, Artificial Sequence
  Oligonucleotide sequence
ugauauuguggggcuuuuctt

SEQ ID NO: 164 - DNA, 21 bp, Artificial Sequence
  Oligonucleotide sequence
gaaaagccccacaauaucatt

SEQ ID NO: 165 - DNA, 21 bp, Artificial Sequence
  Oligonucleotide sequence
gugauauuguggggcuuuutt

SEQ ID NO: 166 - DNA, 21 bp, Artificial Sequence
  Oligonucleotide sequence
aaaagccccacaauaucactt

SEQ ID NO: 167 - DNA, 21 bp, Artificial Sequence
  Oligonucleotide sequence
ggugauauuguggggcuuutt

SEQ ID NO: 168 - DNA, 21 bp, Artificial Sequence
  Oligonucleotide sequence
aaagccccacaauaucacctt

SEQ ID NO: 169 - DNA, 21 bp, Artificial Sequence
  Oligonucleotide sequence
aggugauauuguggggcuutt

SEQ ID NO: 170 - DNA, 21 bp, Artificial Sequence
  Oligonucleotide sequence
aagccccacaauaucaccutt

SEQ ID NO: 171 - DNA, 21 bp, Artificial Sequence
  Oligonucleotide sequence
gggaauagaggugauauugtt

SEQ ID NO: 172 - DNA, 21 bp, Artificial Sequence
  Oligonucleotide sequence
caauaucaccucuauuccctt

SEQ ID NO: 173 - DNA, 21 bp, Artificial Sequence
  Oligonucleotide sequence
ugggaauagaggugauauutt

SEQ ID NO: 174 - DNA, 21 bp, Artificial Sequence
  Oligonucleotide sequence
aauaucaccucuauucccatt

SEQ ID NO: 175 - DNA, 21 bp, Artificial Sequence
  Oligonucleotide sequence
gugggaauagaggugauautt

SEQ ID NO: 176 - DNA, 21 bp, Artificial Sequence
  Oligonucleotide sequence
auaucaccucuauucccactt

SEQ ID NO: 177 - DNA, 21 bp, Artificial Sequence
  Oligonucleotide sequence
agugggaauagaggugauatt

SEQ ID NO: 178 - DNA, 21 bp, Artificial Sequence
  Oligonucleotide sequence
uaucaccucuauucccacutt

SEQ ID NO: 179 - DNA, 21 bp, Artificial Sequence
  Oligonucleotide sequence
cagugggaauagaggugautt

SEQ ID NO: 180 - DNA, 21 bp, Artificial Sequence
  Oligonucleotide sequence
aucaccucuauucccacugtt

SEQ ID NO: 181 - DNA, 21 bp, Artificial Sequence
  Oligonucleotide sequence
ucagugggaauagaggugatt

SEQ ID NO: 182 - DNA, 21 bp, Artificial Sequence
  Oligonucleotide sequence
ucaccucuauucccacugatt

SEQ ID NO: 183 - DNA, 21 bp, Artificial Sequence
  Oligonucleotide sequence
aucagugggaauagaggugtt

SEQ ID NO: 184 - DNA, 21 bp, Artificial Sequence
  Oligonucleotide sequence
caccucuauucccacugautt

SEQ ID NO: 185 - DNA, 21 bp, Artificial Sequence
  Oligonucleotide sequence
gaucagugggaauagaggutt

SEQ ID NO: 186 - DNA, 21 bp, Artificial Sequence
  Oligonucleotide sequence
accucuauucccacugauctt

SEQ ID NO: 187 - DNA, 21 bp, Artificial Sequence
  Oligonucleotide sequence
ggaucagugggaauagaggtt

SEQ ID NO: 188 - DNA, 21 bp, Artificial Sequence
  Oligonucleotide sequence
ccucuauucccacugaucctt

SEQ ID NO: 189 - DNA, 21 bp, Artificial Sequence
  Oligonucleotide sequence
gggaucagugggaauagagtt

SEQ ID NO: 190 - DNA, 21 bp, Artificial Sequence
  Oligonucleotide sequence
cucuauucccacugauccctt

SEQ ID NO: 191 - DNA, 21 bp, Artificial Sequence
  Oligonucleotide sequence
agggaucagugggaauagatt

SEQ ID NO: 192 - DNA, 21 bp, Artificial Sequence
  Oligonucleotide sequence
ucuauucccacugaucccutt

SEQ ID NO: 193 - DNA, 21 bp, Artificial Sequence
  Oligonucleotide sequence
gagggaucagugggaauagtt

SEQ ID NO: 194 - DNA, 21 bp, Artificial Sequence
  Oligonucleotide sequence
cuauucccacugaucccuctt

SEQ ID NO: 195 - DNA, 21 bp, Artificial Sequence
  Oligonucleotide sequence
ugagggaucagugggaauatt

SEQ ID NO: 196 - DNA, 21 bp, Artificial Sequence
  Oligonucleotide sequence
uauucccacugaucccucatt

SEQ ID NO: 197 - DNA, 21 bp, Artificial Sequence
  Oligonucleotide sequence
gugagggaucagugggaautt

SEQ ID NO: 198 - DNA, 21 bp, Artificial Sequence
  Oligonucleotide sequence
auucccacugaucccucactt

SEQ ID NO: 199 - DNA, 21 bp, Artificial Sequence
  Oligonucleotide sequence
agugagggaucagugggaatt

SEQ ID NO: 200 - DNA, 21 bp, Artificial Sequence
  Oligonucleotide sequence
uucccacugaucccucacutt

SEQ ID NO: 201 - DNA, 21 bp, Artificial Sequence
  Oligonucleotide sequence
uagugagggaucagugggatt

SEQ ID NO: 202 - DNA, 21 bp, Artificial Sequence
  Oligonucleotide sequence
ucccacugaucccucacuatt

SEQ ID NO: 203 - DNA, 21 bp, Artificial Sequence
  Oligonucleotide sequence
cuagugagggaucagugggtt

SEQ ID NO: 204 - DNA, 21 bp, Artificial Sequence
  Oligonucleotide sequence
cccacugaucccucacuagtt

SEQ ID NO: 205 - DNA, 21 bp, Artificial Sequence
  Oligonucleotide sequence
accuagugagggaucagugtt

SEQ ID NO: 206 - DNA, 21 bp, Artificial Sequence
  Oligonucleotide sequence
cacugaucccucacuaggutt

SEQ ID NO: 207 - DNA, 21 bp, Artificial Sequence
  Oligonucleotide sequence
gaccuagugagggaucagutt

SEQ ID NO: 208 - DNA, 21 bp, Artificial Sequence
  Oligonucleotide sequence
acugaucccucacuagguctt

SEQ ID NO: 209 - DNA, 21 bp, Artificial Sequence
  Oligonucleotide sequence
ugaccuagugagggaucagtt

SEQ ID NO: 210 - DNA, 21 bp, Artificial Sequence
  Oligonucleotide sequence
cugaucccucacuaggucatt

SEQ ID NO: 211 - DNA, 21 bp, Artificial Sequence
  Oligonucleotide sequence
gugaccuagugagggaucatt

SEQ ID NO: 212 - DNA, 21 bp, Artificial Sequence
  Oligonucleotide sequence
ugaucccucacuaggucactt

SEQ ID NO: 213 - DNA, 21 bp, Artificial Sequence
  Oligonucleotide sequence
ggugaccuagugagggauctt

SEQ ID NO: 214 - DNA, 21 bp, Artificial Sequence
  Oligonucleotide sequence
gaucccucacuaggucacctt

SEQ ID NO: 215 - DNA, 21 bp, Artificial Sequence
  Oligonucleotide sequence
aggugaccuagugagggautt

SEQ ID NO: 216 - DNA, 21 bp, Artificial Sequence
  Oligonucleotide sequence
aucccucacuaggucaccutt

SEQ ID NO: 217 - DNA, 21 bp, Artificial Sequence
  Oligonucleotide sequence
gaggugaccuagugagggatt

SEQ ID NO: 218 - DNA, 21 bp, Artificial Sequence
  Oligonucleotide sequence
ucccucacuaggucaccuctt

SEQ ID NO: 219 - DNA, 21 bp, Artificial Sequence
  Oligonucleotide sequence
ggagaggugaccuagugagtt

SEQ ID NO: 220 - DNA, 21 bp, Artificial Sequence
  Oligonucleotide sequence
cucacuaggucaccucucctt

SEQ ID NO: 221 - DNA, 21 bp, Artificial Sequence
  Oligonucleotide sequence
gggagaggugaccuagugatt

SEQ ID NO: 222 - DNA, 21 bp, Artificial Sequence
  Oligonucleotide sequence
ucacuaggucaccucuccctt

SEQ ID NO: 223 - DNA, 21 bp, Artificial Sequence
  Oligonucleotide sequence
ugggagaggugaccuagugtt

SEQ ID NO: 224 - DNA, 21 bp, Artificial Sequence
  Oligonucleotide sequence
cacuaggucaccucucccatt

SEQ ID NO: 225 - DNA, 21 bp, Artificial Sequence
  Oligonucleotide sequence
cugggagaggugaccuagutt

SEQ ID NO: 226 - DNA, 21 bp, Artificial Sequence
  Oligonucleotide sequence
acuaggucaccucucccagtt

SEQ ID NO: 227 - DNA, 21 bp, Artificial Sequence
  Oligonucleotide sequence
ucugggagaggugaccuagtt

SEQ ID NO: 228 - DNA, 21 bp, Artificial Sequence
  Oligonucleotide sequence
cuaggucaccucucccagatt

SEQ ID NO: 229 - DNA, 21 bp, Artificial Sequence
  Oligonucleotide sequence
uucugggagaggugaccuatt

SEQ ID NO: 230 - DNA, 21 bp, Artificial Sequence
  Oligonucleotide sequence
uaggucaccucucccagaatt

SEQ ID NO: 231 - DNA, 21 bp, Artificial Sequence
  Oligonucleotide sequence
aggugcuccaggugcuucutt

SEQ ID NO: 232 - DNA, 21 bp, Artificial Sequence
  Oligonucleotide sequence
agaagcaccuggagcaccutt

SEQ ID NO: 233 - DNA, 21 bp, Artificial Sequence
  Oligonucleotide sequence
uaggugcuccaggugcuuctt

SEQ ID NO: 234 - DNA, 21 bp, Artificial Sequence
  Oligonucleotide sequence
gaagcaccuggagcaccuatt

SEQ ID NO: 235 - DNA, 21 bp, Artificial Sequence
  Oligonucleotide sequence
ugucuaggugcuccaggugtt

SEQ ID NO: 236 - DNA, 21 bp, Artificial Sequence
  Oligonucleotide sequence
caccuggagcaccuagacatt

SEQ ID NO: 237 - DNA, 21 bp, Artificial Sequence
  Oligonucleotide sequence
ggugucuaggugcuccaggtt

SEQ ID NO: 238 - DNA, 21 bp, Artificial Sequence
  Oligonucleotide sequence
ccuggagcaccuagacacctt

SEQ ID NO: 239 - DNA, 21 bp, Artificial Sequence
  Oligonucleotide sequence
gggugucuaggugcuccagtt

SEQ ID NO: 240 - DNA, 21 bp, Artificial Sequence
  Oligonucleotide sequence
cuggagcaccuagacaccctt

SEQ ID NO: 241 - DNA, 21 bp, Artificial Sequence
  Oligonucleotide sequence
ggggugucuaggugcuccatt

SEQ ID NO: 242 - DNA, 21 bp, Artificial Sequence
  Oligonucleotide sequence
uggagcaccuagacacccctt

SEQ ID NO: 243 - DNA, 21 bp, Artificial Sequence
  Oligonucleotide sequence
uggggugucuaggugcucctt

SEQ ID NO: 244 - DNA, 21 bp, Artificial Sequence
  Oligonucleotide sequence
ggagcaccuagacaccccatt

SEQ ID NO: 245 - DNA, 21 bp, Artificial Sequence
  Oligonucleotide sequence
uuggggugucuaggugcuctt

SEQ ID NO: 246 - DNA, 21 bp, Artificial Sequence
  Oligonucleotide sequence
gagcaccuagacaccccaatt

SEQ ID NO: 247 - DNA, 21 bp, Artificial Sequence
  Oligonucleotide sequence
uuguuggggugucuaggugtt

SEQ ID NO: 248 - DNA, 21 bp, Artificial Sequence
  Oligonucleotide sequence
caccuagacaccccaacaatt

SEQ ID NO: 249 - DNA, 21 bp, Artificial Sequence
  Oligonucleotide sequence
uuuguuggggugucuaggutt

SEQ ID NO: 250 - DNA, 21 bp, Artificial Sequence
  Oligonucleotide sequence
accuagacaccccaacaaatt

SEQ ID NO: 251 - DNA, 21 bp, Artificial Sequence
  Oligonucleotide sequence
cuuuguuggggugucuaggtt

SEQ ID NO: 252 - DNA, 21 bp, Artificial Sequence
  Oligonucleotide sequence
ccuagacaccccaacaaagtt

SEQ ID NO: 253 - DNA, 21 bp, Artificial Sequence
  Oligonucleotide sequence
aguggaccucaauuuccuctt

SEQ ID NO: 254 - DNA, 21 bp, Artificial Sequence
  Oligonucleotide sequence
gaggaaauugagguccacutt

SEQ ID NO: 255 - DNA, 21 bp, Artificial Sequence
  Oligonucleotide sequence
caguggaccucaauuuccutt

SEQ ID NO: 256 - DNA, 21 bp, Artificial Sequence
  Oligonucleotide sequence
aggaaauugagguccacugtt

SEQ ID NO: 257 - DNA, 21 bp, Artificial Sequence
  Oligonucleotide sequence
ucaguggaccucaauuucctt

SEQ ID NO: 258 - DNA, 21 bp, Artificial Sequence
  Oligonucleotide sequence
ggaaauugagguccacugatt

SEQ ID NO: 259 - DNA, 21 bp, Artificial Sequence
  Oligonucleotide sequence
uucaguggaccucaauuuctt

SEQ ID NO: 260 - DNA, 21 bp, Artificial Sequence
  Oligonucleotide sequence
gaaauugagguccacugaatt

SEQ ID NO: 261 - DNA, 21 bp, Artificial Sequence
  Oligonucleotide sequence
guucaguggaccucaauuutt

SEQ ID NO: 262 - DNA, 21 bp, Artificial Sequence
  Oligonucleotide sequence
aaauugagguccacugaactt

SEQ ID NO: 263 - DNA, 21 bp, Artificial Sequence
  Oligonucleotide sequence
aguucaguggaccucaauutt

SEQ ID NO: 264 - DNA, 21 bp, Artificial Sequence
  Oligonucleotide sequence
aauugagguccacugaacutt

SEQ ID NO: 265 - DNA, 21 bp, Artificial Sequence
  Oligonucleotide sequence
aaguucaguggaccucaautt

SEQ ID NO: 266 - DNA, 21 bp, Artificial Sequence
  Oligonucleotide sequence
auugagguccacugaacuutt

SEQ ID NO: 267 - DNA, 21 bp, Artificial Sequence
  Oligonucleotide sequence
uaaguucaguggaccucaatt

SEQ ID NO: 268 - DNA, 21 bp, Artificial Sequence
  Oligonucleotide sequence
uugagguccacugaacuuatt

SEQ ID NO: 269 - DNA, 21 bp, Artificial Sequence
  Oligonucleotide sequence
uuaaguucaguggaccucatt

SEQ ID NO: 270 - DNA, 21 bp, Artificial Sequence
  Oligonucleotide sequence
ugagguccacugaacuuaatt

SEQ ID NO: 271 - DNA, 21 bp, Artificial Sequence
  Oligonucleotide sequence
cuuaaguucaguggaccuctt

SEQ ID NO: 272 - DNA, 21 bp, Artificial Sequence
  Oligonucleotide sequence
gagguccacugaacuuaagtt

SEQ ID NO: 273 - DNA, 21 bp, Artificial Sequence
  Oligonucleotide sequence
acuuaaguucaguggaccutt

SEQ ID NO: 274 - DNA, 21 bp, Artificial Sequence
  Oligonucleotide sequence
agguccacugaacuuaagutt

SEQ ID NO: 275 - DNA, 21 bp, Artificial Sequence
  Oligonucleotide sequence
uacuuaaguucaguggacctt

SEQ ID NO: 276 - DNA, 21 bp, Artificial Sequence
  Oligonucleotide sequence
gguccacugaacuuaaguatt

SEQ ID NO: 277 - DNA, 21 bp, Artificial Sequence
  Oligonucleotide sequence
auacuuaaguucaguggactt

SEQ ID NO: 278 - DNA, 21 bp, Artificial Sequence
  Oligonucleotide sequence
guccacugaacuuaaguautt

SEQ ID NO: 279 - DNA, 21 bp, Artificial Sequence
  Oligonucleotide sequence
gugacaaucaacaacuuugtt

SEQ ID NO: 280 - DNA, 21 bp, Artificial Sequence
  Oligonucleotide sequence
caaaguuguugauugucactt

SEQ ID NO: 281 - DNA, 21 bp, Artificial Sequence
  Oligonucleotide sequence
caugugacaaucaacaacutt

SEQ ID NO: 282 - DNA, 21 bp, Artificial Sequence
  Oligonucleotide sequence
aguuguugauugucacaugtt

SEQ ID NO: 283 - DNA, 21 bp, Artificial Sequence
  Oligonucleotide sequence
gcaugugacaaucaacaactt

SEQ ID NO: 284 - DNA, 21 bp, Artificial Sequence
  Oligonucleotide sequence
guuguugauugucacaugctt

SEQ ID NO: 285 - DNA, 21 bp, Artificial Sequence
  Oligonucleotide sequence
agcaugugacaaucaacaatt

SEQ ID NO: 286 - DNA, 21 bp, Artificial Sequence
  Oligonucleotide sequence
uuguugauugucacaugcutt

SEQ ID NO: 287 - DNA, 21 bp, Artificial Sequence
  Oligonucleotide sequence
aagcaugugacaaucaacatt

SEQ ID NO: 288 - DNA, 21 bp, Artificial Sequence
  Oligonucleotide sequence
uguugauugucacaugcuutt

SEQ ID NO: 289 - DNA, 21 bp, Artificial Sequence
  Oligonucleotide sequence
gaagcaugugacaaucaactt

SEQ ID NO: 290 - DNA, 21 bp, Artificial Sequence
  Oligonucleotide sequence
guugauugucacaugcuuctt

SEQ ID NO: 291 - DNA, 21 bp, Artificial Sequence
  Oligonucleotide sequence
ggaagcaugugacaaucaatt

SEQ ID NO: 292 - DNA, 21 bp, Artificial Sequence
  Oligonucleotide sequence
uugauugucacaugcuucctt

SEQ ID NO: 293 - DNA, 21 bp, Artificial Sequence
  Oligonucleotide sequence
cggaagcaugugacaaucatt

SEQ ID NO: 294 - DNA, 21 bp, Artificial Sequence
  Oligonucleotide sequence
ugauugucacaugcuuccgtt

SEQ ID NO: 295 - DNA, 21 bp, Artificial Sequence
  Oligonucleotide sequence
ccggaagcaugugacaauctt

SEQ ID NO: 296 - DNA, 21 bp, Artificial Sequence
  Oligonucleotide sequence
gauugucacaugcuuccggtt

SEQ ID NO: 297 - DNA, 21 bp, Artificial Sequence
  Oligonucleotide sequence
cccggaagcaugugacaautt

SEQ ID NO: 298 - DNA, 21 bp, Artificial Sequence
  Oligonucleotide sequence
auugucacaugcuuccgggtt

SEQ ID NO: 299 - DNA, 21 bp, Artificial Sequence
  Oligonucleotide sequence
ucccggaagcaugugacaatt

SEQ ID NO: 300 - DNA, 21 bp, Artificial Sequence
  Oligonucleotide sequence
uugucacaugcuuccgggatt

SEQ ID NO: 301 - DNA, 21 bp, Artificial Sequence
  Oligonucleotide sequence
uucccggaagcaugugacatt

SEQ ID NO: 302 - DNA, 21 bp, Artificial Sequence
  Oligonucleotide sequence
ugucacaugcuuccgggaatt

SEQ ID NO: 303 - DNA, 21 bp, Artificial Sequence
  Oligonucleotide sequence
cuucccggaagcaugugactt

SEQ ID NO: 304 - DNA, 21 bp, Artificial Sequence
  Oligonucleotide sequence
gucacaugcuuccgggaagtt

SEQ ID NO: 305 - DNA, 21 bp, Artificial Sequence
  Oligonucleotide sequence
ccuucccggaagcaugugatt

SEQ ID NO: 306 - DNA, 21 bp, Artificial Sequence
  Oligonucleotide sequence
ucacaugcuuccgggaaggtt

SEQ ID NO: 307 - DNA, 21 bp, Artificial Sequence
  Oligonucleotide sequence
uccuucccggaagcaugugtt

SEQ ID NO: 308 - DNA, 21 bp, Artificial Sequence
  Oligonucleotide sequence
cacaugcuuccgggaaggatt

SEQ ID NO: 309 - DNA, 21 bp, Artificial Sequence
  Oligonucleotide sequence
cuccuucccggaagcaugutt

SEQ ID NO: 310 - DNA, 21 bp, Artificial Sequence
  Oligonucleotide sequence
acaugcuuccgggaaggagtt

SEQ ID NO: 311 - DNA, 21 bp, Artificial Sequence
  Oligonucleotide sequence
ccuccuucccggaagcaugtt

SEQ ID NO: 312 - DNA, 21 bp, Artificial Sequence
  Oligonucleotide sequence
caugcuuccgggaaggaggtt

SEQ ID NO: 313 - DNA, 21 bp, Artificial Sequence
  Oligonucleotide sequence
cccuccuucccggaagcautt

SEQ ID NO: 314 - DNA, 21 bp, Artificial Sequence
  Oligonucleotide sequence
augcuuccgggaaggagggtt

SEQ ID NO: 315 - DNA, 21 bp, Artificial Sequence
  Oligonucleotide sequence
ucccuccuucccggaagcatt

SEQ ID NO: 316 - DNA, 21 bp, Artificial Sequence
  Oligonucleotide sequence
ugcuuccgggaaggagggatt

SEQ ID NO: 317 - DNA, 21 bp, Artificial Sequence
  Oligonucleotide sequence
auucccuccuucccggaagtt

SEQ ID NO: 318 - DNA, 21 bp, Artificial Sequence
  Oligonucleotide sequence
cuuccgggaaggagggaautt

SEQ ID NO: 319 - DNA, 21 bp, Artificial Sequence
  Oligonucleotide sequence
aauucccuccuucccggaatt

SEQ ID NO: 320 - DNA, 21 bp, Artificial Sequence
  Oligonucleotide sequence
uuccgggaaggagggaauutt

SEQ ID NO: 321 - DNA, 21 bp, Artificial Sequence
  Oligonucleotide sequence
ucuccaauucccuccuucctt

SEQ ID NO: 322 - DNA, 21 bp, Artificial Sequence
  Oligonucleotide sequence
ggaaggagggaauuggagatt

SEQ ID NO: 323 - DNA, 21 bp, Artificial Sequence
  Oligonucleotide sequence
cucuccaauucccuccuuctt

SEQ ID NO: 324 - DNA, 21 bp, Artificial Sequence
  Oligonucleotide sequence
gaaggagggaauuggagagtt

SEQ ID NO: 325 - DNA, 21 bp, Artificial Sequence
  Oligonucleotide sequence
ucucuccaauucccuccuutt

SEQ ID NO: 326 - DNA, 21 bp, Artificial Sequence
  Oligonucleotide sequence
aaggagggaauuggagagatt

SEQ ID NO: 327 - DNA, 21 bp, Artificial Sequence
  Oligonucleotide sequence
gucucuccaauucccuccutt

SEQ ID NO: 328 - DNA, 21 bp, Artificial Sequence
  Oligonucleotide sequence
aggagggaauuggagagactt

SEQ ID NO: 329 - DNA, 21 bp, Artificial Sequence
  Oligonucleotide sequence
agucucuccaauucccucctt

SEQ ID NO: 330 - DNA, 21 bp, Artificial Sequence
  Oligonucleotide sequence
ggagggaauuggagagacutt

SEQ ID NO: 331 - DNA, 21 bp, Artificial Sequence
  Oligonucleotide sequence
uagucucuccaauucccuctt

SEQ ID NO: 332 - DNA, 21 bp, Artificial Sequence
  Oligonucleotide sequence
gagggaauuggagagacuatt

SEQ ID NO: 333 - DNA, 21 bp, Artificial Sequence
  Oligonucleotide sequence
guagucucuccaauucccutt

SEQ ID NO: 334 - DNA, 21 bp, Artificial Sequence
  Oligonucleotide sequence
agggaauuggagagacuactt

SEQ ID NO: 335 - DNA, 21 bp, Artificial Sequence
  Oligonucleotide sequence
gguagucucuccaauuccctt

SEQ ID NO: 336 - DNA, 21 bp, Artificial Sequence
  Oligonucleotide sequence
gggaauuggagagacuacctt

SEQ ID NO: 337 - DNA, 21 bp, Artificial Sequence
  Oligonucleotide sequence
ugcaaccacagggauuucutt

SEQ ID NO: 338 - DNA, 21 bp, Artificial Sequence
  Oligonucleotide sequence
agaaaucccugugguugcatt

SEQ ID NO: 339 - DNA, 21 bp, Artificial Sequence
  Oligonucleotide sequence
cugcaaccacagggauuuctt

SEQ ID NO: 340 - DNA, 21 bp, Artificial Sequence
  Oligonucleotide sequence
gaaaucccugugguugcagtt

SEQ ID NO: 341 - DNA, 21 bp, Artificial Sequence
  Oligonucleotide sequence
gcugcaaccacagggauuutt

SEQ ID NO: 342 - DNA, 21 bp, Artificial Sequence
  Oligonucleotide sequence
aaaucccugugguugcagctt

SEQ ID NO: 343 - DNA, 21 bp, Artificial Sequence
  Oligonucleotide sequence
ugcugcaaccacagggauutt

SEQ ID NO: 344 - DNA, 21 bp, Artificial Sequence
  Oligonucleotide sequence
aaucccugugguugcagcatt

SEQ ID NO: 345 - DNA, 21 bp, Artificial Sequence
  Oligonucleotide sequence
cugcugcaaccacagggautt

SEQ ID NO: 346 - DNA, 21 bp, Artificial Sequence
  Oligonucleotide sequence
aucccugugguugcagcagtt

SEQ ID NO: 347 - DNA, 21 bp, Artificial Sequence
  Oligonucleotide sequence
gcugcugcaaccacagggatt

SEQ ID NO: 348 - DNA, 21 bp, Artificial Sequence
  Oligonucleotide sequence
ucccugugguugcagcagctt

SEQ ID NO: 349 - DNA, 21 bp, Artificial Sequence
  Oligonucleotide sequence
agcugcugcaaccacagggtt

SEQ ID NO: 350 - DNA, 21 bp, Artificial Sequence
  Oligonucleotide sequence
cccugugguugcagcagcutt

SEQ ID NO: 351 - DNA, 21 bp, Artificial Sequence
  Oligonucleotide sequence
aaagcugcugcaaccacagtt

SEQ ID NO: 352 - DNA, 21 bp, Artificial Sequence
  Oligonucleotide sequence
cugugguugcagcagcuuutt

SEQ ID NO: 353 - DNA, 21 bp, Artificial Sequence
  Oligonucleotide sequence
caaagcugcugcaaccacatt

SEQ ID NO: 354 - DNA, 21 bp, Artificial Sequence
  Oligonucleotide sequence
ugugguugcagcagcuuugtt

SEQ ID NO: 355 - DNA, 21 bp, Artificial Sequence
  Oligonucleotide sequence
acaaagcugcugcaaccactt

SEQ ID NO: 356 - DNA, 21 bp, Artificial Sequence
  Oligonucleotide sequence
gugguugcagcagcuuugutt

SEQ ID NO: 357 - DNA, 21 bp, Artificial Sequence
  Oligonucleotide sequence
aacaaagcugcugcaaccatt

SEQ ID NO: 358 - DNA, 21 bp, Artificial Sequence
  Oligonucleotide sequence
ugguugcagcagcuuuguutt

SEQ ID NO: 359 - DNA, 21 bp, Artificial Sequence
  Oligonucleotide sequence
caacaaagcugcugcaacctt

SEQ ID NO: 360 - DNA, 21 bp, Artificial Sequence
  Oligonucleotide sequence
gguugcagcagcuuuguugtt

SEQ ID NO: 361 - DNA, 21 bp, Artificial Sequence
  Oligonucleotide sequence
ccaacaaagcugcugcaactt

SEQ ID NO: 362 - DNA, 21 bp, Artificial Sequence
  Oligonucleotide sequence
guugcagcagcuuuguuggtt

SEQ ID NO: 363 - DNA, 21 bp, Artificial Sequence
  Oligonucleotide sequence
gccaacaaagcugcugcaatt

SEQ ID NO: 364 - DNA, 21 bp, Artificial Sequence
  Oligonucleotide sequence
uugcagcagcuuuguuggctt

SEQ ID NO: 365 - DNA, 21 bp, Artificial Sequence
  Oligonucleotide sequence
ggccaacaaagcugcugcatt

SEQ ID NO: 366 - DNA, 21 bp, Artificial Sequence
  Oligonucleotide sequence
ugcagcagcuuuguuggcctt

SEQ ID NO: 367 - DNA, 21 bp, Artificial Sequence
  Oligonucleotide sequence
uggccaacaaagcugcugctt

SEQ ID NO: 368 - DNA, 21 bp, Artificial Sequence
  Oligonucleotide sequence
gcagcagcuuuguuggccatt

SEQ ID NO: 369 - DNA, 21 bp, Artificial Sequence
  Oligonucleotide sequence
cuggccaacaaagcugcugtt

SEQ ID NO: 370 - DNA, 21 bp, Artificial Sequence
  Oligonucleotide sequence
cagcagcuuuguuggccagtt

SEQ ID NO: 371 - DNA, 21 bp, Artificial Sequence
  Oligonucleotide sequence
ccuggccaacaaagcugcutt

SEQ ID NO: 372 - DNA, 21 bp, Artificial Sequence
  Oligonucleotide sequence
agcagcuuuguuggccaggtt

SEQ ID NO: 373 - DNA, 21 bp, Artificial Sequence
  Oligonucleotide sequence
uuccuggccaacaaagcugtt

SEQ ID NO: 374 - DNA, 21 bp, Artificial Sequence
  Oligonucleotide sequence
cagcuuuguuggccaggaatt

SEQ ID NO: 375 - DNA, 21 bp, Artificial Sequence
  Oligonucleotide sequence
cuuccuggccaacaaagcutt

SEQ ID NO: 376 - DNA, 21 bp, Artificial Sequence
  Oligonucleotide sequence
agcuuuguuggccaggaagtt

SEQ ID NO: 377 - DNA, 21 bp, Artificial Sequence
  Oligonucleotide sequence
cccuuccuggccaacaaagtt

SEQ ID NO: 378 - DNA, 21 bp, Artificial Sequence
  Oligonucleotide sequence
cuuuguuggccaggaagggtt

SEQ ID NO: 379 - DNA, 21 bp, Artificial Sequence
  Oligonucleotide sequence
ccccuuccuggccaacaaatt

SEQ ID NO: 380 - DNA, 21 bp, Artificial Sequence
  Oligonucleotide sequence
uuuguuggccaggaaggggtt

SEQ ID NO: 381 - DNA, 21 bp, Artificial Sequence
  Oligonucleotide sequence
uccccuuccuggccaacaatt

SEQ ID NO: 382 - DNA, 21 bp, Artificial Sequence
  Oligonucleotide sequence
uuguuggccaggaaggggatt

SEQ ID NO: 383 - DNA, 21 bp, Artificial Sequence
  Oligonucleotide sequence
cuccccuuccuggccaacatt

SEQ ID NO: 384 - DNA, 21 bp, Artificial Sequence
  Oligonucleotide sequence
uguuggccaggaaggggagtt

SEQ ID NO: 385 - DNA, 21 bp, Artificial Sequence
  Oligonucleotide sequence
uccuccccuuccuggccaatt

SEQ ID NO: 386 - DNA, 21 bp, Artificial Sequence
  Oligonucleotide sequence
uuggccaggaaggggaggatt

SEQ ID NO: 387 - DNA, 21 bp, Artificial Sequence
  Oligonucleotide sequence
auccuccccuuccuggccatt

SEQ ID NO: 388 - DNA, 21 bp, Artificial Sequence
  Oligonucleotide sequence
uggccaggaaggggaggautt

SEQ ID NO: 389 - DNA, 21 bp, Artificial Sequence
  Oligonucleotide sequence
ucaaauccuccccuuccugtt

SEQ ID NO: 390 - DNA, 21 bp, Artificial Sequence
  Oligonucleotide sequence
caggaaggggaggauuugatt

SEQ ID NO: 391 - DNA, 21 bp, Artificial Sequence
  Oligonucleotide sequence
gucaaauccuccccuuccutt

SEQ ID NO: 392 - DNA, 21 bp, Artificial Sequence
  Oligonucleotide sequence
aggaaggggaggauuugactt

SEQ ID NO: 393 - DNA, 21 bp, Artificial Sequence
  Oligonucleotide sequence
cgucaaauccuccccuucctt

SEQ ID NO: 394 - DNA, 21 bp, Artificial Sequence
  Oligonucleotide sequence
ggaaggggaggauuugacgtt

SEQ ID NO: 395 - DNA, 21 bp, Artificial Sequence
  Oligonucleotide sequence
ucgucaaauccuccccuuctt

SEQ ID NO: 396 - DNA, 21 bp, Artificial Sequence
  Oligonucleotide sequence
gaaggggaggauuugacgatt

SEQ ID NO: 397 - DNA, 21 bp, Artificial Sequence
  Oligonucleotide sequence
cucgucaaauccuccccuutt

SEQ ID NO: 398 - DNA, 21 bp, Artificial Sequence
  Oligonucleotide sequence
aaggggaggauuugacgagtt

SEQ ID NO: 399 - DNA, 21 bp, Artificial Sequence
  Oligonucleotide sequence
acucgucaaauccuccccutt

SEQ ID NO: 400 - DNA, 21 bp, Artificial Sequence
  Oligonucleotide sequence
aggggaggauuugacgagutt

SEQ ID NO: 401 - DNA, 21 bp, Artificial Sequence
  Oligonucleotide sequence
ucacucgucaaauccuccctt

SEQ ID NO: 402 - DNA, 21 bp, Artificial Sequence
  Oligonucleotide sequence
gggaggauuugacgagugatt

SEQ ID NO: 403 - DNA, 21 bp, Artificial Sequence
  Oligonucleotide sequence
cucacucgucaaauccucctt

SEQ ID NO: 404 - DNA, 21 bp, Artificial Sequence
  Oligonucleotide sequence
ggaggauuugacgagugagtt

SEQ ID NO: 405 - DNA, 21 bp, Artificial Sequence
  Oligonucleotide sequence
acucacucgucaaauccuctt

SEQ ID NO: 406 - DNA, 21 bp, Artificial Sequence
  Oligonucleotide sequence
gaggauuugacgagugagutt

SEQ ID NO: 407 - DNA, 21 bp, Artificial Sequence
  Oligonucleotide sequence
caacucacucgucaaaucctt

SEQ ID NO: 408 - DNA, 21 bp, Artificial Sequence
  Oligonucleotide sequence
ggauuugacgagugaguugtt

SEQ ID NO: 409 - DNA, 21 bp, Artificial Sequence
  Oligonucleotide sequence
acaacucacucgucaaauctt

SEQ ID NO: 410 - DNA, 21 bp, Artificial Sequence
  Oligonucleotide sequence
gauuugacgagugaguugutt

SEQ ID NO: 411 - DNA, 21 bp, Artificial Sequence
  Oligonucleotide sequence
gacaacucacucgucaaautt

SEQ ID NO: 412 - DNA, 21 bp, Artificial Sequence
  Oligonucleotide sequence
auuugacgagugaguuguctt

SEQ ID NO: 413 - DNA, 21 bp, Artificial Sequence
  Oligonucleotide sequence
agacaacucacucgucaaatt

SEQ ID NO: 414 - DNA, 21 bp, Artificial Sequence
  Oligonucleotide sequence
uuugacgagugaguugucutt

SEQ ID NO: 415 - DNA, 21 bp, Artificial Sequence
  Oligonucleotide sequence
cagacaacucacucgucaatt

SEQ ID NO: 416 - DNA, 21 bp, Artificial Sequence
  Oligonucleotide sequence
uugacgagugaguugucugtt

SEQ ID NO: 417 - DNA, 21 bp, Artificial Sequence
  Oligonucleotide sequence
acagacaacucacucgucatt

SEQ ID NO: 418 - DNA, 21 bp, Artificial Sequence
  Oligonucleotide sequence
ugacgagugaguugucugutt

SEQ ID NO: 419 - DNA, 21 bp, Artificial Sequence
  Oligonucleotide sequence
gacagacaacucacucguctt

SEQ ID NO: 420 - DNA, 21 bp, Artificial Sequence
  Oligonucleotide sequence
gacgagugaguugucuguctt

SEQ ID NO: 421 - DNA, 21 bp, Artificial Sequence
  Oligonucleotide sequence
agacagacaacucacucgutt

SEQ ID NO: 422 - DNA, 21 bp, Artificial Sequence
  Oligonucleotide sequence
acgagugaguugucugucutt

SEQ ID NO: 423 - DNA, 21 bp, Artificial Sequence
  Oligonucleotide sequence
gagacagacaacucacucgtt

SEQ ID NO: 424 - DNA, 21 bp, Artificial Sequence
  Oligonucleotide sequence
cgagugaguugucugucuctt

SEQ ID NO: 425 - DNA, 21 bp, Artificial Sequence
  Oligonucleotide sequence
ggagacagacaacucacuctt

SEQ ID NO: 426 - DNA, 21 bp, Artificial Sequence
  Oligonucleotide sequence
gagugaguugucugucucctt

SEQ ID NO: 427 - DNA, 21 bp, Artificial Sequence
  Oligonucleotide sequence
aggagacagacaacucacutt

SEQ ID NO: 428 - DNA, 21 bp, Artificial Sequence
  Oligonucleotide sequence
agugaguugucugucuccutt

SEQ ID NO: 429 - DNA, 21 bp, Artificial Sequence
  Oligonucleotide sequence
caggagacagacaacucactt

SEQ ID NO: 430 - DNA, 21 bp, Artificial Sequence
  Oligonucleotide sequence
gugaguugucugucuccugtt

SEQ ID NO: 431 - DNA, 21 bp, Artificial Sequence
  Oligonucleotide sequence
ucaggagacagacaacucatt

SEQ ID NO: 432 - DNA, 21 bp, Artificial Sequence
  Oligonucleotide sequence
ugaguugucugucuccugatt

SEQ ID NO: 433 - DNA, 21 bp, Artificial Sequence
  Oligonucleotide sequence
uucaggagacagacaacuctt

SEQ ID NO: 434 - DNA, 21 bp, Artificial Sequence
  Oligonucleotide sequence
gaguugucugucuccugaatt

SEQ ID NO: 435 - DNA, 21 bp, Artificial Sequence
  Oligonucleotide sequence
auucaggagacagacaacutt

SEQ ID NO: 436 - DNA, 21 bp, Artificial Sequence
  Oligonucleotide sequence
aguugucugucuccugaautt

SEQ ID NO: 437 - DNA, 21 bp, Artificial Sequence
  Oligonucleotide sequence
uauucaggagacagacaactt

SEQ ID NO: 438 - DNA, 21 bp, Artificial Sequence
  Oligonucleotide sequence
guugucugucuccugaauatt

SEQ ID NO: 439 - DNA, 21 bp, Artificial Sequence
  Oligonucleotide sequence
guauucaggagacagacaatt

SEQ ID NO: 440 - DNA, 21 bp, Artificial Sequence
  Oligonucleotide sequence
uugucugucuccugaauactt

SEQ ID NO: 441 - DNA, 21 bp, Artificial Sequence
  Oligonucleotide sequence
aguauucaggagacagacatt

SEQ ID NO: 442 - DNA, 21 bp, Artificial Sequence
  Oligonucleotide sequence
ugucugucuccugaauacutt

SEQ ID NO: 443 - DNA, 21 bp, Artificial Sequence
  Oligonucleotide sequence
gaguauucaggagacagactt

SEQ ID NO: 444 - DNA, 21 bp, Artificial Sequence
  Oligonucleotide sequence
gucugucuccugaauacuctt

SEQ ID NO: 445 - DNA, 21 bp, Artificial Sequence
  Oligonucleotide sequence
ggaguauucaggagacagatt

SEQ ID NO: 446 - DNA, 21 bp, Artificial Sequence
  Oligonucleotide sequence
ucugucuccugaauacucctt

SEQ ID NO: 447 - DNA, 21 bp, Artificial Sequence
  Oligonucleotide sequence
gggaguauucaggagacagtt

SEQ ID NO: 448 - DNA, 21 bp, Artificial Sequence
  Oligonucleotide sequence
cugucuccugaauacuccctt

SEQ ID NO: 449 - DNA, 21 bp, Artificial Sequence
  Oligonucleotide sequence
ggggaguauucaggagacatt

SEQ ID NO: 450 - DNA, 21 bp, Artificial Sequence
  Oligonucleotide sequence
ugucuccugaauacucccctt

SEQ ID NO: 451 - DNA, 21 bp, Artificial Sequence
  Oligonucleotide sequence
uggggaguauucaggagactt

SEQ ID NO: 452 - DNA, 21 bp, Artificial Sequence
  Oligonucleotide sequence
gucuccugaauacuccccatt

SEQ ID NO: 453 - DNA, 21 bp, Artificial Sequence
  Oligonucleotide sequence
guggggaguauucaggagatt

SEQ ID NO: 454 - DNA, 21 bp, Artificial Sequence
  Oligonucleotide sequence
ucuccugaauacuccccactt

SEQ ID NO: 455 - DNA, 21 bp, Artificial Sequence
  Oligonucleotide sequence
uguggggaguauucaggagtt

SEQ ID NO: 456 - DNA, 21 bp, Artificial Sequence
  Oligonucleotide sequence
cuccugaauacuccccacatt

SEQ ID NO: 457 - DNA, 21 bp, Artificial Sequence
  Oligonucleotide sequence
auguggggaguauucaggatt

SEQ ID NO: 458 - DNA, 21 bp, Artificial Sequence
  Oligonucleotide sequence
uccugaauacuccccacautt

SEQ ID NO: 459 - DNA, 21 bp, Artificial Sequence
  Oligonucleotide sequence
uauguggggaguauucaggtt

SEQ ID NO: 460 - DNA, 21 bp, Artificial Sequence
  Oligonucleotide sequence
ccugaauacuccccacauatt

SEQ ID NO: 461 - DNA, 21 bp, Artificial Sequence
  Oligonucleotide sequence
cuauguggggaguauucagtt

SEQ ID NO: 462 - DNA, 21 bp, Artificial Sequence
  Oligonucleotide sequence
cugaauacuccccacauagtt

SEQ ID NO: 463 - DNA, 21 bp, Artificial Sequence
  Oligonucleotide sequence
gcuauguggggaguauucatt

SEQ ID NO: 464 - DNA, 21 bp, Artificial Sequence
  Oligonucleotide sequence
ugaauacuccccacauagctt

SEQ ID NO: 465 - DNA, 21 bp, Artificial Sequence
  Oligonucleotide sequence
ggcuauguggggaguauuctt

SEQ ID NO: 466 - DNA, 21 bp, Artificial Sequence
  Oligonucleotide sequence
gaauacuccccacauagcctt

SEQ ID NO: 467 - DNA, 21 bp, Artificial Sequence
  Oligonucleotide sequence
gggcuauguggggaguauutt

SEQ ID NO: 468 - DNA, 21 bp, Artificial Sequence
  Oligonucleotide sequence
aauacuccccacauagccctt

SEQ ID NO: 469 - DNA, 1003 bp, Homo sapiens
gcaggaggcaaaagtcctgtgttccaactatagtcatttctttgctgcatgatctgagttaggtcaccagacttctctgagccccagtttccccagcagtgtatacgggctatgtggggagtattcaggagacagacaactcactcgtcaaatcctccccttcctggccaacaaagctgctgcaaccacagggatttcttctgttcaggtgagtgtagggtgtagggagattggttcaatgtccaattcttctgtttccctggagatcaggttgcccttttttggtagtctctccaattccctccttcccggaagcatgtgacaatcaacaactttgtatacttaagttcagtggacctcaatttcctcatctgtgaaataaacgggactgaaaaatcattctggcctcaagatgctttgttggggtgtctaggtgctccaggtgcttctgggagaggtgacctagtgagggatcagtgggaatagaggtgatattgtggggcttttctggaaattgcagagaggtgcatcgtttttataatttatgaatttttatgtattaatgtcatcctcctgatcttttcagctgcattgggtaaatccttgcctgccagagtgggtcagcggtgagccagaaagggggctcattctaacagtgctgtgtcctcctggagagtgccaactcattctccaagtaaaaaaagccagatttgtggctcacttcgtggggaaatgtgtccagcgcaccaacgcaggcgagggactgggggaggagggaagtgccctcctgcagcacgcgaggttccgggaccggctggcctgctggaactcggccaggctcagctggctcggcgctgggcagccaggagcctgggccccggggagggcggtcccgggcggcgcggtgggccgagcgcgggtcccgcctccttgaggcgggcccgggcggggcggttgtatatcagggccgcgctgagctgcgccagctgaggtgtgagcagct

SEQ ID NO: 470 - DNA, 50 bp, Artificial Sequence
  Primer sequence
gtcgtatccagtgcagggtccgaggtattcgcactggatacgactgccaa

SEQ ID NO: 471 - DNA, 23 bp, Artificial Sequence
  Primer sequence
cgcgtatacttggagaatgagtt

SEQ ID NO: 472 - DNA, 16 bp, Artificial Sequence
  Primer sequence
gtgcagggtccgaggt

SEQ ID NO: 473 - DNA, 20 bp, Artificial Sequence
  Primer sequence
ccaggtgatgcccttctgta

SEQ ID NO: 474 - DNA, 20 bp, Artificial Sequence
  Primer sequence
gagcaactcacagtcacgct

SEQ ID NO: 475 - DNA, 24 bp, Artificial Sequence
  Primer sequence
gatagttaagtgggatcgagacat

SEQ ID NO: 476 - DNA, 21 bp, Artificial Sequence
  Primer sequence
agcaagcaagcagaatttgga

SEQ ID NO: 477 - DNA, 21 bp, Artificial Sequence
  Oligonucleotide sequence
acuacugagugacaguagatt

SEQ ID NO: 478 - DNA, 21 bp, Artificial Sequence
  Oligonucleotide sequence
ucuacugucacucaguagutt

SEQ ID NO: 479 - RNA, 19 nt, Artificial Sequence
  Oligonucleotide sequence
ccaacucauucuccaaguc

SEQ ID NO: 480 - RNA, 22 nt, Artificial Sequence
  Oligonucleotide sequence
uacuuggagaaugaguuggcac

SEQ ID NO: 481 - RNA, 19 nt, Artificial Sequence
  Oligonucleotide sequence
ccaacucauucuccaaguc

SEQ ID NO: 482 - RNA, 21 nt, Artificial Sequence
  Oligonucleotide sequence
uacuuggagaaugaguuggca

SEQ ID NO: 483 - DNA, 21 bp, Artificial Sequence
  Oligonucleotide sequence
uucugggagaggugaccuatt

SEQ ID NO: 484 - DNA, 21 bp, Artificial Sequence
  Oligonucleotide sequence
uaggucaccucucccagaatt

SEQ ID NO: 485 - DNA, 21 bp, Artificial Sequence
  Oligonucleotide sequence
gggaguauucaggagacagtt

SEQ ID NO: 486 - DNA, 21 bp, Artificial Sequence
  Oligonucleotide sequence
cugucuccugaauacuccctt

SEQ ID NO: 487 - RNA, 19 nt, Artificial Sequence
  Oligonucleotide sequence
  modified_base (1)..(19): (1,2,18,19) = 2'-O-methyl
  modified_base (6)..(12): (6,9,10,12) = 2'-fluoro
  modified_base (17)..(19): (17,18,19) = phosphorothioate (PS) backbone modification
ccaacucauucuccaaguc

SEQ ID NO: 488 - RNA, 21 nt, Artificial Sequence
  Oligonucleotide sequence
  modified_base (1)..(21): (1,3,4,5,12,16,17,20,21) = 2'-fluoro
  modified_base (19)..(21): (19,20,21) = phosphorothioate (PS) backbone modification
uacuuggagaaugaguuggca

SEQ ID NO: 489 - RNA, 19 nt, Artificial Sequence
  Oligonucleotide sequence
  modified_base (1)..(19): (1,2,18,19) = 2'-O-methyl
  modified_base (1)..(1): (1) = Linked to cholesterol conjugate(s) via Triethylene glycol linker (Chol-TEG)
  modified_base (6)..(12): (6,9,10,12) = 2'-fluoro
  modified_base (17)..(19): (17,18,19) = phosphorothioate (PS) backbone modification
ccaacucauucuccaaguc

SEQ ID NO: 490 - RNA, 19 nt, Artificial Sequence
  Oligonucleotide sequence
  modified_base (1)..(19): (1,2,18,19) = 2'-O-methyl
  modified_base (1)..(1): (1) = Linked to cholesterol conjugate(s) via Triethylene glycol linker (Chol-TEG)
  modified_base (6)..(12): (6,9,10,12) = 2'-fluoro
  modified_base (17)..(19): (17,18,19) = phosphorothioate (PS) backbone modification
cuagcucguucuuccaugc

SEQ ID NO: 491 - RNA, 21 nt, Artificial Sequence
  Oligonucleotide sequence
  modified_base (1)..(21): (1,3,4,5,12,16,17,20,21) = 2'-fluoro
  modified_base (19)..(21): (19,20,21) = phosphorothioate (PS) backbone modification
ucauggaagaacgagcuagca

SEQ ID NO: 492 - RNA, 21 nt, Artificial Sequence
  Oligonucleotide sequence
  modified_base (1)..(21): (1,2,3,19,20,21) = phosphorothioate (PS) backbone modification
  modified_base (1)..(21): (1,3,5,7,9,10,11,13,15,17,19,21) = 2'-fluoro
  modified_base (2)..(20): (2,4,6,8,12,14,16,18,20) = 2'-O-methyl
cgacuacugagugacaguaga

SEQ ID NO: 493 - RNA, 23 nt, Artificial Sequence
  Oligonucleotide sequence
  modified_base (1)..(23): (1,2,3,19,21,22,23) = phosphorothioate (PS) backbone modification
  modified_base (1)..(23): (3,5,7,9,11,13,15,17,19,21,23) = 2'-O-methyl
  modified_base (1)..(1): (1) = 5'(E)-vinylphosphonate
  modified_base (2)..(22): (2,4,6,8,10,12,14,16,18,20,22) = 2'-fluoro
ucuacugucacucaguagucguc

SEQ ID NO: 494 - RNA, 21 nt, Artificial Sequence
  Oligonucleotide sequence
gucaucacacugaauaccaau

SEQ ID NO: 495 - RNA, 23 nt, Artificial Sequence
  Oligonucleotide sequence
auugguauucagugugaugacac

SEQ ID NO: 496 - RNA, 21 nt, Artificial Sequence
  Oligonucleotide sequence
ugccaacucauucuccaagua

SEQ ID NO: 497 - RNA, 23 nt, Artificial Sequence
  Oligonucleotide sequence
uacuuggagaaugaguuggcacu

SEQ ID NO: 498 - RNA, 21 nt, Artificial Sequence
  Oligonucleotide sequence
  modified_base (1)..(21): (1,2,3,19,20,21) = phosphorothioate (PS) backbone modification
  modified_base (1)..(21): (1,3,5,7,9,10,11,13,15,17,19,21) = 2'-fluoro
  modified_base (2)..(20): (2,4,6,8,12,14,16,18,20) = 2'-O-methyl
ugccaacucauucuccaagua

SEQ ID NO: 499 - RNA, 23 nt, Artificial Sequence
  Oligonucleotide sequence
  modified_base (1)..(23): (1,2,3,21,22,23) = phosphorothioate (PS) backbone modification
  modified_base (1)..(23): (1,3,5,7,9,11,13,15,17,19,21,23) = 2'-O-methyl
  modified_base (2)..(22): (2,4,6,8,10,12,14,16,18,20,22) = 2'-fluoro
uacuuggagaaugaguuggcacu

SEQ ID NO: 500 - RNA, 23 nt, Artificial Sequence
  Oligonucleotide sequence
  modified_base (1)..(23): (1,2,3,19,21,22,23) = phosphorothioate (PS) backbone modification
  modified_base (1)..(23): (3,5,7,9,11,13,15,17,19,21,23) = 2'-O-methyl
  modified_base (1)..(1): (1) = 5'-(E)-vinylphosphonate
  modified_base (2)..(22): (2,4,6,8,10,12,14,16,18,20,22) = 2'-fluoro
uacuuggagaaugaguuggcacu

SEQ ID NO: 501 - RNA, 21 nt, Artificial Sequence
  Oligonucleotide sequence
  modified_base (1)..(21): (1,2,3,19,20,21) = phosphorothioate (PS) backbone modification
  modified_base (1)..(21): (1,3,5,7,9,10,11,13,15,17,19,21) = 2'-fluoro
  modified_base (2)..(20): (2,4,6,8,12,14,16,18,20) = 2'-O-methyl
  modified_base (21)..(21): (21) = Linked to  liposome structure group via a controlled microporous glass
ugccaacucauucuccaagua

SEQ ID NO: 502 - DNA, 21 bp, Artificial Sequence
  Oligonucleotide sequence
agugccaacucauucuccatt

SEQ ID NO: 503 - DNA, 21 bp, Artificial Sequence
  Oligonucleotide sequence
uggagaaugaguuggcacutt

SEQ ID NO: 504 - DNA, 21 bp, Artificial Sequence
  Oligonucleotide sequence
gagugccaacucauucucctt

SEQ ID NO: 505 - DNA, 21 bp, Artificial Sequence
  Oligonucleotide sequence
ggagaaugaguuggcacuctt

SEQ ID NO: 506 - DNA, 21 bp, Artificial Sequence
  Oligonucleotide sequence
agagugccaacucauucuctt

SEQ ID NO: 507 - DNA, 21 bp, Artificial Sequence
  Oligonucleotide sequence
gagaaugaguuggcacucutt

SEQ ID NO: 508 - DNA, 21 bp, Artificial Sequence
  Oligonucleotide sequence
gagagugccaacucauucutt

SEQ ID NO: 509 - DNA, 21 bp, Artificial Sequence
  Oligonucleotide sequence
agaaugaguuggcacucuctt

SEQ ID NO: 510 - DNA, 21 bp, Artificial Sequence
  Oligonucleotide sequence
ggagagugccaacucauuctt

SEQ ID NO: 511 - DNA, 21 bp, Artificial Sequence
  Oligonucleotide sequence
gaaugaguuggcacucucctt